European Patent Specification EP 3 207 139 B1, published May 7, 2025. Title: METHODS AND COMPOSITIONS FOR MULTIPLEX RNA GUIDED GENOME EDITING AND OTHER RNA TECHNOLOGIES. Applicant: Penn State University Research Foundation. The sequence listing filed with the application follows.

SEQUENCE LISTING (189 sequences)

SEQ ID NO: 1 - DNA, 113 bp, Artificial Sequence
  sgRNA1 target MPK5
gatccgtggcaagatgtcgtagagcaggtacgttttagagctagaaatagcaagttaaaataaggctagtccgttatcaacttgaaaaagtggcaccgagtcggtgctttttt

SEQ ID NO: 2 - DNA, 115 bp, Artificial Sequence
  sgRNA2 target MPK5
gatccgtggcagtctacatcgccacggagctcagttttagagctagaaatagcaagttaaaataaggctagtccgttatcaacttgaaaaagtggcaccgagtcggtgctttttt

SEQ ID NO: 3 - DNA, 96 bp, Artificial Sequence
  gRNA1 scaffold target MPK5
agatgtcgtagagcaggtacgttttagagctagaaatagcaagttaaaataaggctagtccgttatcaacttgaaaaagtggcaccgagtcggtgc

SEQ ID NO: 4 - DNA, 97 bp, Artificial Sequence
  gRNA2 scaffold target MPK5
tctacatcgccacggagctcagttttagagctagaaatagcaagttaaaataaggctagtccgttatcaacttgaaaaagtggcaccgagtcggtgc

SEQ ID NO: 5 - DNA, 96 bp, Artificial Sequence
  gRNA3 scaffold. Target MPK1
atccaggcgacgctgagccagttttagagctagaaatagcaagttaaaataaggctagtccgttatcaacttgaaaaagtggcaccgagtcggtgc

SEQ ID NO: 6 - DNA, 96 bp, Artificial Sequence
  gRNA4 scaffold. Target MPK1
tggcccaccggggtataaaagttttagagctagaaatagcaagttaaaataaggctagtccgttatcaacttgaaaaagtggcaccgagtcggtgc

SEQ ID NO: 7 - DNA, 96 bp, Artificial Sequence
  gRNA5 scaffold. Target MPK2
gaacccggtcgcctcaaggagttttagagctagaaatagcaagttaaaataaggctagtccgttatcaacttgaaaaagtggcaccgagtcggtgc

SEQ ID NO: 8 - DNA, 96 bp, Artificial Sequence
  gRNA6 scaffold. Target MPK2
gaatgcgcagactcgtcagggttttagagctagaaatagcaagttaaaataaggctagtccgttatcaacttgaaaaagtggcaccgagtcggtgc

SEQ ID NO: 9 - DNA, 96 bp, Artificial Sequence
  gRNA7 scaffold. Target MPK6
gtgtccgcttggcatcgatagttttagagctagaaatagcaagttaaaataaggctagtccgttatcaacttgaaaaagtggcaccgagtcggtgc

SEQ ID NO: 10 - DNA, 96 bp, Artificial Sequence
  gRNA8 scaffold. Target MPK6
gcgggtgcgggtcaatcaaagttttagagctagaaatagcaagttaaaataaggctagtccgttatcaacttgaaaaagtggcaccgagtcggtgc

SEQ ID NO: 11 - DNA, 96 bp, Artificial Sequence
  gRNA9 scaffold. Target PDS
acaagccaggagaattcagcgttttagagctagaaatagcaagttaaaataaggctagtccgttatcaacttgaaaaagtggcaccgagtcggtgc

SEQ ID NO: 12 - DNA, 96 bp, Artificial Sequence
  gRNA10 scaffold. Target PDS
cactgcatggataactcatcgttttagagctagaaatagcaagttaaaataaggctagtccgttatcaacttgaaaaagtggcaccgagtcggtgc

SEQ ID NO: 13 - DNA, 77 bp, Artificial Sequence
  pre-tRNA sequence
aacaaagcaccagtggtctagtggtggaatagtaccctgccacggtacagacccgggttcgattcccggctggtgca

SEQ ID NO: 14 - DNA, 10 bp, Artificial Sequence
  Last 10bp of U3 promoter
gatccgtggc

SEQ ID NO: 15 - DNA, 153 bp, Artificial Sequence
  gRNA-tRNA in pGTR plasmid
gttttagagctagaaatagcaagttaaaataaggctagtccgttatcaacttgaaaaagtggcaccgagtcggtgcaacaaagcaccagtggtctagtggtagaatagtaccctgccacggtacagacccgggttcgattcccggctggtgca

SEQ ID NO: 16 - DNA, 193 bp, Artificial Sequence
  tRNA-gRNA1
gatccgtggcaacaaagcaccagtggtctagtggtagaatagtaccctgccacggtacagacccgggttcgattcccggctggtgcaagatgtcgtagagcaggtacgttttagagctagaaatagcaagttaaaataaggctagtccgttatcaacttgaaaaagtggcaccgagtcggtgctttttttttt

SEQ ID NO: 17 - DNA, 194 bp, Artificial Sequence
  tRNA-gRNA2
gatccgtggcaacaaagcaccagtggtctagtggtagaatagtaccctgccacggtacagacccgggttcgattcccggctggtgcatctacatcgccacggagctcagttttagagctagaaatagcaagttaaaataaggctagtccgttatcaacttgaaaaagtggcaccgagtcggtgctttttttttt

SEQ ID NO: 18 - DNA, 270 bp, Artificial Sequence
  tRNA-gRNA1-tRNA
gatccgtggcaacaaagcaccagtggtctagtggtagaatagtaccctgccacggtacagacccgggttcgattcccggctggtgcaagatgtcgtagagcaggtacgttttagagctagaaatagcaagttaaaataaggctagtccgttatcaacttgaaaaagtggcaccgagtcggtgcaacaaagcaccagtggtctagtggtagaatagtaccctgccacggtacagacccgggttcgattcccggctggtgcatttttttttt

SEQ ID NO: 19 - DNA, 271 bp, Artificial Sequence
  tRNA-gRNA2-tRNA
gatccgtggcaacaaagcaccagtggtctagtggtagaatagtaccctgccacggtacagacccgggttcgattcccggctggtgcatctacatcgccacggagctcagttttagagctagaaatagcaagttaaaataaggctagtccgttatcaacttgaaaaagtggcaccgagtcggtgcaacaaagcaccagtggtctagtggtagaatagtaccctgccacggtacagacccgggttcgattcccggctggtgcatttttttttt

SEQ ID NO: 20 - DNA, 365 bp, Artificial Sequence
  tRNA-gRNA3-tRNA-gRNA4
gatccgtggcaacaaagcaccagtggtctagtggtagaatagtaccctgccacggtacagacccgggttcgattcccggctggtgcaatccaggcgacgctgagccagttttagagctagaaatagcaagttaaaataaggctagtccgttatcaacttgaaaaagtggcaccgagtcggtgcaacaaagcaccagtggtctagtggtagaatagtaccctgccacggtacagacccgggttcgattcccggctggtgcatggcccaccggggtataaaagttttagagctagaaatagcaagttaaaataaggctagtccgttatcaacttgaaaaagtggcaccgagtcggtgcttttttttt

SEQ ID NO: 21 - DNA, 366 bp, Artificial Sequence
  tRNA-gRNA5-tRNA-gRNA6
gatccgtggcaacaaagcaccagtggtctagtggtagaatagtaccctgccacggtacagacccgggttcgattcccggctggtgcagaacccggtcgcctcaaggagttttagagctagaaatagcaagttaaaataaggctagtccgttatcaacttgaaaaagtggcaccgagtcggtgcaacaaagcaccagtggtctagtggtagaatagtaccctgccacggtacagacccgggttcgattcccggctggtgcagaatgcgcagactcgtcagggttttagagctagaaatagcaagttaaaataaggctagtccgttatcaacttgaaaaagtggcaccgagtcggtgctttttttttt

SEQ ID NO: 22 - DNA, 366 bp, Artificial Sequence
  tRNA-gRNA7-tRNA-gRNA8
gatgatccgtggcaacaaagcaccagtggtctagtggtagaatagtaccctgccacggtacagacccgggttcgattcccggctggtgcagtgtccgcttggcatcgatagttttagagctagaaatagcaagttaaaataaggctagtccgttatcaacttgaaaaagtggcaccgagtcggtgcaacaaagcaccagtggtctagtggtagaatagtaccctgccacggtacagacccgggttcgattcccggctggtgcagcgggtgcgggtcaatcaaagttttagagctagaaatagcaagttaaaataaggctagtccgttatcaacttgaaaaagtggcaccgagtcggtgcttttttt

SEQ ID NO: 23 - DNA, 367 bp, Artificial Sequence
  tRNA-gRNA1-tRNA-gRNA2
gatccgtggcaacaaagcaccagtggtctagtggtagaatagtaccctgccacggtacagacccgggttcgattcccggctggtgcaagatgtcgtagagcaggtacgttttagagctagaaatagcaagttaaaataaggctagtccgttatcaacttgaaaaagtggcaccgagtcggtgcaacaaagcaccagtggtctagtggtagaatagtaccctgccacggtacagacccgggttcgattcccggctggtgcatctacatcgccacggagctcagttttagagctagaaatagcaagttaaaataaggctagtccgttatcaacttgaaaaagtggcaccgagtcggtgctttttttttt

SEQ ID NO: 24 - DNA, 713 bp, Artificial Sequence
  tRNA-gRNA1-tRNA-gRNA2-tRNA-gRNA3-tRNA-gRNA4
gatccgtggcaataaagcaccagtggtctagtggtagaatagtaccctgccacggtacagacccgggttcgattcccggctggtgcaagatgtcgtagagcaggtacgttttagagctagaaatagcaagttaaaataaggctagtccgttatcaacttgaaaaagtggcaccgagtcggtgcaacaaagcaccagtggtctagtggtagaatagtaccctgccacggtacagacccgggttcgattcccggctggtgcatctacatcgccacggagctcagttttagagctagaaatagcaagttaaaataaggctagtccgttatcaacttgaaaaagtggcaccgagtcggtgcaacaaagcaccagtggtctagtggtagaatagtaccctgccacggtacagacccgggttcgattcccggctggtgcaatccaggcgacgctgagccagttttagagctagaaatagcaagttaaaataaggctagtccgttatcaacttgaaaaagtggcaccgagtcggtgcaacaaagcaccagtggtctagtggtagaatagtaccctgccacggtacagacccgggttcgattcccggctggtgcatggcccaccggggtataaaagttttagagctagaaatagcaagttaaaataaggctagtccgttatcaacttgaaaaagtggcaccgagtcggtgctttttttttt

SEQ ID NO: 25 - DNA, 711 bp, Artificial Sequence
  tRNA-gRNA7-tRNA-gRNA8-tRNA-gRNA5-tRNA-gRNA6
gatccgtggcaacaaagcaccagtggtctagtggtagaatagtaccctgccacggtacagacccgggttcgattcccggctggtgcagtgtccgcttggcatcgatagttttagagctagaaatagcaagttaaaataaggctagtccgttatcaacttgaaaaagtggcaccgagtcggtgcaacaaagcaccagtggtctagtggtagaatagtaccctgccacggtacagacccgggttcgattcccggctggtgcagcgggtgcgggtcaatcaaagttttagagctagaaatagcaagttaaaataaggctagtccgttatcaacttgaaaaagtggcaccgagtcggtgcaacaaagcaccagtggtctagtggtagaatagtaccctgccacggtacagacccgggttcgattcccggctggtgcagaacccggtcgcctcaaggagttttagagctagaaatagcaagttaaaataaggctagtccgttatcaacttgaaaaagtggcaccgagtcggtgcaacaaagcaccagtggtctagtggtagaatagtaccctgccacggtacagacccgggttcgattcccggctggtgcagaatgcgcagactcgtcagggttttagagctagaaatagcaagttaaaataaggctagtccgttatcaacttgaaaaagtggcaccgagtcggtgcttttttttt

SEQ ID NO: 26 - DNA, 1404 bp, Artificial Sequence
  tRNA-gRNA1-tRNA-gRNA2-tRNA-gRNA3-tRNA-gRNA4-tRNA-gRNA7-tRNA-gRNA8 -tRNA-gRNA5-tRNA-gRNA6
gatccgtggcaacaaagcaccagtggtctagtggtagaatagtaccctgccacggtacagacccgggttcgattcccggctggtgcaagatgtcgtagagcaggtacgttttagagctagaaatagcaagttaaaataaggctagtccgttatcaacttgaaaaagtggcaccgagtcggtgcaacaaagcaccagtggtctagtggtagaatagtaccctgccacggtacagacccgggttcgattcccggctggtgcatctacatcgccacggagctcagttttagagctagaaatagcaagttaaaataaggctagtccgttatcaacttgaaaaagtggcaccgagtcggtgcaacaaagcaccagtggtctagtggtagaatagtaccctgccacggtacagacccgggttcgattcccggctggtgcaatccaggcgacgctgagccagttttagagctagaaatagcaagttaaaataaggctagtccgttatcaacttgaaaaagtggcaccgagtcggtgcaacaaagcaccagtggtctagtggtagaatagtaccctgccacggtacagacccgggttcgattcccggctggtgcatggcccaccggggtataaaagttttagagctagaaatagcaagttaaaataaggctagtccgttatcaacttgaaaaagtggcaccgagtcggtgcaacaaagcaccagtggtctagtggtagaatagtaccctgccacggtacagacccgggttcgattcccggctggtgcagtgtccgcttggcatcgatagttttagagctagaaatagcaagttaaaataaggctagtccgttatcaacttgaaaaagtggcaccgagtcggtgcaacaaagcaccagtggtctagtggtagaatagtaccctgccacggtacagacccgggttcgattcccggctggtgcagcgggtgcgggtcaatcaaagttttagagctagaaatagcaagttaaaataaggctagtccgttatcaacttgaaaaagcggcaccgagtcggtgcaacaaagcaccagtggtctagtggtagaatagtaccctgccacggtacagacccgggttcgattcccggctggtgcagaacccggtcgcctcaaggagttttagagctagaaatagcaagttaaaataaggctagtccgttatcaacttgaaaaagtggcaccgagtcggtgcaacaaagcaccagtggtctagtggtagaatagtaccctgccacggtacagacccgggttcgattcccggctggtgcagaatgcgcagactcgtcagggttttagagctagaaatagcaagttaaaataaggctagtccgttatcaacttgaaaaagtggcaccgagtcggtgcttttttttt

SEQ ID NO: 27 - DNA, 367 bp, Artificial Sequence
  tRNA-gRNA9-tRNA-gRNA10
gatccgtggcaacaaagcaccagtggtctagtggtggaatagtaccctgccacggtacagacccgggttcgattcccggctggtgcaacaagccaggagaattcagcgttttagagctagaaatagcaagttaaaataaggctagtccgttatcaacttgaaaaagtggcaccgagtcggtgcaacaaagcaccagtggtctagtggtagaatagtaccctgccacggtacagacccgggtccgattcccggctggtgcacactgcatggataactcatcgttttagagctagaaatagcaagttaaaataaggctagtccgttatcaacttgaaaaagtggcaccgagtcggtgcttttttttttt

SEQ ID NO: 28 - DNA, 20 bp, Artificial Sequence
  Primer gRNA1-R for cRT-PCR of gRNA1
aaacgtacctgctctacgac

SEQ ID NO: 29 - DNA, 20 bp, Artificial Sequence
  Primer gRNA2-R for cRT-PCR of gRNA2
aaactgagctccgtggcgat

SEQ ID NO: 30 - DNA, 34 bp, Artificial Sequence
  Primer Bsa-gRNA-F for cRT-PCR and amplify gRNA
ggagaccgaggtctcggttttagagctagaaata

SEQ ID NO: 31 - DNA, 24 bp, Artificial Sequence
  Primer gRNA1-F for qRT-PCR
ggcaagatgtcgtagagcaggtac

SEQ ID NO: 32 - DNA, 22 bp, Artificial Sequence
  Primer gRNA2-F for qRT-PCR
gtctacatcgccacggagctca

SEQ ID NO: 33 - DNA, 18 bp, Artificial Sequence
  Primer gRNA-R for qRT-PCR
gcaccgactcggtgccac

SEQ ID NO: 34 - DNA, 22 bp, Artificial Sequence
  Primer UBI-qF for qRT-PCR
tggtcagtaatcagccagtttg

SEQ ID NO: 35 - DNA, 22 bp, Artificial Sequence
  Primer UBI-qR for qRT-PCR
caaatacttgacgaacagaggc

SEQ ID NO: 36 - DNA, 20 bp, Artificial Sequence
  Primer MPK5-qF for qPCR
gatcccgccgccgatccctc

SEQ ID NO: 37 - DNA, 54 bp, Artificial Sequence
  Primer g-tRNA-F for construct pGTR
gcaccgagtcggtgcaacaaagcaccagtggtctagtggtagaatagtaccctg

SEQ ID NO: 38 - DNA, 60 bp, Artificial Sequence
  Primer tRNA-R for construct pGTR
ctgccatgcaccagccgggaatcgaacccgggtctgtaccgtggcagggtactattctac

SEQ ID NO: 39 - DNA, 37 bp, Artificial Sequence
  Primer UBI-F for amplifying UBIp
tgcatgcctgcaggtccacaaattcgggtcaaggcgg

SEQ ID NO: 40 - DNA, 41 bp, Artificial Sequence
  Primer UBI-R to amplify UBIp
caaacttgttgataactatctgcaagaaataatcaccaaac

SEQ ID NO: 41 - DNA, 41 bp, Artificial Sequence
  Primer UGW-U3-F for construct pRGE32
gaccatgattacgccaagcttaaggaatctttaaacatacg

SEQ ID NO: 42 - DNA, 37 bp, Artificial Sequence
  Primer UGW-gRNA-R for construct pRGE32
ggacctgcaggcatgcacgcgctaaaaacggactagc

SEQ ID NO: 43 - DNA, 18 bp, Artificial Sequence
  Primer MPK1-F for Genotyping of MPK1
gggtcggcacagcatctc

SEQ ID NO: 44 - DNA, 20 bp, Artificial Sequence
  Primer MPK1-R2 for genotyping of MPK1
tgcgcctaaaaatcgagggt

SEQ ID NO: 45 - DNA, 21 bp, Artificial Sequence
  Primer  MPK2-F for genotyping of MPK2
tttgggaagcatgtatgaagc

SEQ ID NO: 46 - DNA, 20 bp, Artificial Sequence
  Primer MPK2-R2 for genotyping of MPK2
tatgccagccaatgagccaa

SEQ ID NO: 47 - DNA, 21 bp, Artificial Sequence
  Primer MPK5-F256 for genotyping of MPK5
gccaccttccttcctcatccg

SEQ ID NO: 48 - DNA, 20 bp, Artificial Sequence
  Primer MPK5-R611 for genotyping of MPK5
gttgctcggcttcaggtcgc

SEQ ID NO: 49 - DNA, 21 bp, Artificial Sequence
  Primer MPK6-F for genotyping of MPK6
ttgacgccccaacataaataa

SEQ ID NO: 50 - DNA, 18 bp, Artificial Sequence
  Primer MPK6-R for genotyping of MPK6
tgttgctgccgcttttct

SEQ ID NO: 51 - DNA, 20 bp, Artificial Sequence
  Primer PDS-F for genotyping of PDS
ggtagaaatgccatgcggga

SEQ ID NO: 52 - DNA, 20 bp, Artificial Sequence
  Primer PDS-R for genotyping of PDS
attcagccgaacctcaccac

SEQ ID NO: 53 - DNA, 46 bp, Artificial Sequence
  Primer  L5AD5-F for PTG synthesis and cloning
cgggtctcaggcaggatgggcagtctgggcaacaaagcaccagtgg

SEQ ID NO: 54 - DNA, 52 bp, Artificial Sequence
  Primer L3AD5-R for PTG synthesis and cloning
taggtctccaaacggatgagcgacagcaaacaaaaaaaaaagcaccgactcg

SEQ ID NO: 55 - DNA, 31 bp, Artificial Sequence
  Primer S5AD5-F for PTG synthesis and cloning
cgggtctcaggcaggatgggcagtctgggca

SEQ ID NO: 56 - DNA, 31 bp, Artificial Sequence
  Primer S3AD5-R for PTG synthesis and cloning
taggtctccaaacggatgagcgacagcaaac

SEQ ID NO: 57 - DNA, 36 bp, Artificial Sequence
  Primer gR1-F for synthesis of PTG
taggtctcctagagcaggtacgttttagagctagaa

SEQ ID NO: 58 - DNA, 36 bp, Artificial Sequence
  Primer gR1-R for synthesis of PTG
atggtctcatctacgacatcttgcaccagccgggaa

SEQ ID NO: 59 - DNA, 36 bp, Artificial Sequence
  Primer gR2-F for synthesis of PTG
taggtctccccacggagctcagttttagagctagaa

SEQ ID NO: 60 - DNA, 37 bp, Artificial Sequence
  Primer gR2-R for synthesis of PTG
atggtctcagtggcgatgtagatgcaccagccgggaa

SEQ ID NO: 61 - DNA, 36 bp, Artificial Sequence
  Primer gR3-F for synthesis of PTG
taggtctccgacgctgagccagttttagagctagaa

SEQ ID NO: 62 - DNA, 36 bp, Artificial Sequence
  Primer gR3-R for synthesis of PTG
atggtctcacgtcgcctggattgcaccagccgggaa

SEQ ID NO: 63 - DNA, 38 bp, Artificial Sequence
  Primer gR4-F for synthesis of PTG
taggtctccaccggggtataaaagttttagagctagaa

SEQ ID NO: 64 - DNA, 32 bp, Artificial Sequence
  Primer gR4-R  for synthesis of PTG
cgggtctcacggtgggccatgcaccagccggg

SEQ ID NO: 65 - DNA, 37 bp, Artificial Sequence
  Primer gR5-F for synthesis of PTG
taggtctccgtcgcctcaaggagttttagagctagaa

SEQ ID NO: 66 - DNA, 33 bp, Artificial Sequence
  Primer gR5-R for synthesis of PTG
cgggtctcacgaccgggttctgcaccagccggg

SEQ ID NO: 67 - DNA, 37 bp, Artificial Sequence
  Primer gR6-F for synthesis of PTG
taggtctcccagactcgtcagggttttagagctagaa

SEQ ID NO: 68 - DNA, 33 bp, Artificial Sequence
  Primer gR6-R for synthesis of PTG
cgggtctcatctgcgcattctgcaccagccggg

SEQ ID NO: 69 - DNA, 36 bp, Artificial Sequence
  Primer gR7-F for synthesis of PTG
taggtctccttggcatcgatagttttagagctagaa

SEQ ID NO: 70 - DNA, 36 bp, Artificial Sequence
  Primer  gR7-R for synthesis of PTG
atggtctcaccaagcggacactgcaccagccgggaa

SEQ ID NO: 71 - DNA, 37 bp, Artificial Sequence
  Primer gR8-F for synthesis of PTG
taggtctcccgggtcaatcaaagttttagagctagaa

SEQ ID NO: 72 - DNA, 33 bp, Artificial Sequence
  Primer gR8-R for synthesis of PTG
cgggtctcacccgcacccgctgcaccagccggg

SEQ ID NO: 73 - DNA, 21 bp, Artificial Sequence
  Primer Ln-gR7-F for synthesis of PTG
taggtctccttggcatcgata

SEQ ID NO: 74 - DNA, 21 bp, Artificial Sequence
  Primer Ln-gR7-R for synthesis of PTG
atggtctcaccaagcggacac

SEQ ID NO: 75 - DNA, 38 bp, Artificial Sequence
  Primer gR9-F for synthesis of PTG
taggtctcccaggagaattcagcgttttagagctagaa

SEQ ID NO: 76 - DNA, 32 bp, Artificial Sequence
  Primer gR9-R for synthesis of PTG
cgggtctcacctggcttgttgcaccagccggg

SEQ ID NO: 77 - DNA, 38 bp, Artificial Sequence
  Primer gR10-F Artificial synthesis of PTG
taggtctccatggataactcatcgttttagagctagaa

SEQ ID NO: 78 - DNA, 32 bp, Artificial Sequence
  Primer gR10-R for synthesis of PTG
cgggtctcaccatgcagtgtgcaccagccggg

SEQ ID NO: 79 - DNA, 1720 bp, Oryza sativa
attccgcctccactttcccttcccttcctcctccacctccacctcctcgtcgcgatccaaatccgaatccggccatggacgccggggcgcagccgccggacacggagatggcggaggccggcggcgggcagcagccgcctgctgcggctgcggcggcgggggcgggggcaggggcggggatgatggagaacatccaggcgacgctgagccatggcgggaggttcatccagtacaacatcttcgggaacgtgttcgaggtcaccgccaagtacaagccccccatcctccccatcggcaagggcgcctacggcatcgtctgctcggcgctcaactcggagacgggggagcaggtggcgatcaagaagatcgccaacgcgttcgacaacaagatcgacgccaagcgcacgctcagggagatcaagctgctccgccacatggaccacgagaatattgttgccataagggatatcatacctcctccacaaaggaattcattcaatgacgtttatattgcatatgaattgatggatactgatctgcatcaaattattcgctcaaatcaagcattgtcagaggagcactgccagtatttcctttatcagattctccgtggcttgaagtatatacattcagcaaatgtccttcaccgagacttgaagcccagcaacctacttttgaatgcaaattgtgacctcaaaatttgtgattttggacttgctcgtaccacctcagaaaccgattttatgactgagtatgttgtcacaagatggtatagggcaccggaacttctgttgaattcctctgaatatactgcagcaattgatgtgtggtctgtgggctgtatttttatggaactcatggatcgtaaacctttgtttcctggaagagatcatgtccatcaattacgtctactaatggagctcatcggaacgccaaatgaggctgatctggattttgtaaatgaaaatgcaagaagatacattcgccaacttcctagacatgcaaggcagtcctttcctgaaaaatttccacatgttcatcctttagcaattgatctggttgaaaagatgctgacatttgatcctagacagagaataacagttgaaggtgcccttgcacatccttacctggcatcactgcatgacataagtgatgagccagtctgctcatcacccttcagctttgacttcgagcagcatgcattgtccgaggaacaaatgaaggatctaatctaccaagaaggccttgcgttcaaccctgattaccagtagctggtgttctatttcagccttggattgattctattcatatggagttttttcctcctgcgccacaaaaggtcgccgacagtgatcactagttgtaaataattgcctcacctgaaaaatcctccctggttcaaagctgaaggtgttgttctaagagtagaaatgtactttgtgatcaagttcctgggtagctgctatgccattcttatgcttatgtatgttgtttaatgtgggatttttttccatcttaaatgtttttagtcccttttgtaagaagagttagttcatgaacgatgacggcctaaattctgcggttatcatcaaattccccattttcttgtcgattcatggatttctcatggttttacttaatgctccatgttgtaagacgtggtcaatggaagaggatatattgactcttgattcagtggtggcagtttggagttgatcgt

SEQ ID NO: 80 - protein, 398 aa, Oryza sativa
MDAGAQPPDTEMAEAGGGQQPPAAAAAAGAGAGAGMMENIQATLSHGGRFIQYNIFGNVFEVTAKYKPPILPIGKGAYGIVCSALNSETGEQVAIKKIANAFDNKIDAKRTLREIKLLRHMDHENIVAIRDIIPPPQRNSFNDVYIAYELMDTDLHQIIRSNQALSEEHCQYFLYQILRGLKYIHSANVLHRDLKPSNLLLNANCDLKICDFGLARTTSETDFMTEYVVTRWYRAPELLLNSSEYTAAIDVWSVGCIFMELMDRKPLFPGRDHVHQLRLLMELIGTPNEADLDFVNENARRYIRQLPRHARQSFPEKFPHVHPLAIDLVEKMLTFDPRQRITVEGALAHPYLASLHDISDEPVCSSPFSFDFEQHALSEEQMKDLIYQEGLAFNPDYQ

SEQ ID NO: 81 - DNA, 1577 bp, Oryza sativa
gggttcgtttcttggctggttttcttgggcggcgatcgatcgatgcgcatggagggcggcggcggcggcggccatggccatcacggcggcggcggcggtggccatggccatcacggtggcatcggaggaggggaggcgcagatcaaggggacgctgacgcacggcgggaggtacgtgcagtacaacgtgtatggtaacctgttcgaggtttcgtccaagtacgtccctcccatccgccccgtcggccgcggcgcctgcggcatcatctgtgcggttgtgaatgcgcagactcgtcaggaggtggcaatcaagaagatcggcaacgcgttcgacaaccagatcgacgccaagcgcaccctgcgagagatcaagctgcttcggcacatggatcatgataatgtcatctcaataaaggacatcatacggccaccaaggagggagaacttcaatgatgtctacattgtctatgagctcatggacactgatcttcaccaccttcttcgatcaaaccagccactaacagatgatcactgtcagtattttctctatcaggtactacgaggattgaagtatgtgcattcagcaaatgtcttgcacagagacctcaggccaagtaatttgctgctgaatgcgaaatgcgatcttaagatcggagactttggattagcaaggaccacaaatgaaactgacttcatgatggagtatgttgttactcgatggtacagggcacctgaactcctgctaaactgctcagagtacactgcagctattgatatctggtcggtaggctgcatccttggtgagatcgttacaagggagcctttgtttcctggaaaggattatgtccatcagctgaggctaataactgagttaataggctcacctgatgactcgagccttgggtttcttcgaagcgacaacgcccgcagatatgtgaggtcgcttcctcaataccccaagcaacaattccgtgcacggttccccactatgtctagtggtgccatggatttgcttgagaggatgcttgtgtttgatcccagcaaaaggattactgttgatgaagctctgtgccatccatacttggcatcccttcatgagatatatgatgaaccagtctgcccagcgcctttcagcttcgatttcgagcagccgtcgctcaccgaagaagatatcaaggagatcatatggagggaggcacttaagttcaaccctgaaccaattcactagatgaatttccaatgaagaacggaagcagatcacactggcagatgatcatccatccactccttggggaagacatgagccaacagcatgatgtatagttgatcaccctctcagcatctcatcttgtggcttgtcagcgacaccctgacatcgcaaattcggacatttatgaaaacaagaaaagcttgatcaaataatttgtagtacgaaaaaaatcaggagcttaactgtatcttcttgttagatttgtatctatcccatttggttgtatgcttaagaaacctgggagcttgtcactagttatggaggtacagcaatctccagatactcttcagtcatcagttcagttcacc

SEQ ID NO: 82 - DNA, 1489 bp, Oryza sativa
agcgatcacaaattgtgccaattcacaaaccgccgcccccttccctttttaatagctgccttcgcctctcgtcccctctccctcatcgccttgctgtctctgcgaatcgagagagagtcagataaggtcgttaattaggtttgtcaattcggctgcttgcggcgagagaagaggaggagggattagggatggacggggcgccggtggcggagttcaggccgacgatgacgcacggcggccggtacctgctctacgacatcttcgggaacaagttcgaggtgacgaacaagtaccagccgcccatcatgcccattggccgcggcgcctacgggatcgtctgctccgtgatgaactttgagacgagggagatggtggcgataaagaagatcgccaacgcgttcaacaacgacatggacgccaagcgcacgctccgggagatcaagctcctcaggcacctcgaccacgagaacatcataggcatcagggatgtgatcccgccgccgatccctcaggcgttcaacgacgtctacatcgccacggagctcatggacaccgacctccatcacatcatccgctccaaccaagaactgtcagaagagcactgccagtatttcctgtaccagatcctgcgggggctcaagtacatccactcggcgaacgtgatccaccgcgacctgaagccgagcaacctgctgctgaacgccaactgcgacctcaagatctgcgacttcgggctggcgcggccgtcgtcggagagcgacatgatgacggagtacgtggtcacccggtggtaccgcgcgccggagctgctgctcaactccaccgactactccgccgccatcgacgtctggtccgtcggctgcatcttcatggagctcatcaaccgccagccgctcttccccggcagggaccacatgcaccagatgcgcctcatcaccgaggtgatcgggacgccgacggacgacgagctggggttcatacggaacgaggacgcgaggaagtacatgaggcacctgccgcagtacccgcgccggacgttcgcgagcatgttcccgcgggtgcagcccgccgcgctcgacctcatcgagaggatgctcaccttcaacccgctgcagagaatcacagttgaggaggcgctcgatcatccttacctagagagattgcacgacatcgccgatgagcccatctgcctggagcccttctccttcgacttcgagcagaaggctctaaacgaggaccaaatgaagcagctgatcttcaacgaagcgatcgagatgaacccaaacatccggtactagattgaatcaccatggaaatgagatcccgtctatacctgctttgtacatatgatcaagattgagagccgggtagactgaacattgcatttgtttgtttgttgatgttcgaaacccacattctctgcaagttgtggctgctttgtatgatatatggtactatgttcgaataaaagggtttggaactttggatt

SEQ ID NO: 83 - protein, 369 aa, Oryza sativa
MDGAPVAEFRPTMTHGGRYLLYDIFGNKFEVTNKYQPPIMPIGRGAYGIVCSVMNFETREMVAIKKIANAFNNDMDAKRTLREIKLLRHLDHENIIGIRDVIPPPIPQAFNDVYIATELMDTDLHHIIRSNQELSEEHCQYFLYQILRGLKYIHSANVIHRDLKPSNLLLNANCDLKICDFGLARPSSESDMMTEYVVTRWYRAPELLLNSTDYSAAIDVWSVGCIFMELINRQPLFPGRDHMHQMRLITEVIGTPTDDELGFIRNEDARKYMRHLPQYPRRTFASMFPRVQPAALDLIERMLTFNPLQRITVEEALDHPYLERLHDIADEPICLEPFSFDFEQKALNEDQMKQLIFNEAIEMNPNIRY

SEQ ID NO: 84 - DNA, 1560 bp, Oryza sativa
attccgcggtcgccgcccgagtcaaaaagagggggaagcttctcccaccatagtcctcctcctcctcctcctactcccatcaacgactagtcgcggcgaccaagagccaaaccctacgcctcctcccctccccctccacctcgtcctccccgcgagcggcggcggccatggattcctcctccggcggcgcgggcggcggcggcggcgcgcagatcaaggggatggggacgcacgggggccgctacgtgctgtacaacgtgtacgggaacttcttcgaggtctcctccaagtacgcccctcccatccgccccatcggccggggcgcctacggcattgtctgcgcggctgttaactcggagaacggcgaggaagttgccatcaagaagattggcaatgcattcgacaaccatatcgatgccaagcggacactgagagaaatcaagctgcttcgccacatggaccacgagaatattattgccataaaggacataattcgccccccaagaagagacaactttaatgatgtttacattgtttctgagttgatggatactgatctccatcagatcatacgctcaaatcaaccattgactgatgaccactgccagtacttcctgtaccagttgctacgagggctaaaatatgtgcactcggcaaatgtcttgcaccgtgatctgaagccaagcaatttgttccttaatgcaaattgtgatctcaagattgctgattttgggcttgcaagaaccactacggagactgacctcatgacagagtatgtggtcactcgttggtatcgagcaccagagctgctgttgaactgctcgcagtatactgctgctattgatgtctggtcagttggatgcatacttggtgaaattgtgactcgtcaacccctgtttcctggaagggattacattcagcaactaaaattgatcactgagctgatagggtcgccagatgactcaagcctagggtttcttcggagtgataatgcaagaagatacatgaaacagctaccacagtacccaaggcaggacttccgcttgcgcttccgcaacatgtctgctggtgcagtcgatctgttagagaaaatgctggtgtttgacccaagcagacggataactgttgatgaggctcttcatcacccatacttggcttctcttcatgacatcaatgaagaacccacctgcccagcacctttcagctttgattttgagcaaccatcctttactgaagaacatataaaagaactcatctggagggaatccttggcatttaatccggatcctccctactaagagctcagagcaatttatcaatgctggcatctgaagatcggtagctctagaaaagccaaatccccttgctttgtgcatctattaattttatgcccacttgttgggcgaatgagcatggattattgttatagtgacaatttttcttaaggcctgtctaaagaaacaacatttgtattccttatcagatagcctgaacttgggcctgtattataccggttgattgcataactgttcttatgtatctaagcctgtaattgtcttc

SEQ ID NO: 85 - DNA, 1641 bp, Oryza sativa
gcatcagctccacccccgaaaaatttctccccaatctcgcgaggctctcgtcgtcgaatcgaatcctctcgcgtcctcaagatgcagatctttgtgaagacattgaccggcaagactatcaccctcgaggtggagtcctctgacaccatcgataatgtcaaggctaagatccaagataaggagggcatccccccggaccagcagcgtctcatcttcgctggcaagcagctggaggatggcaggacccttgctgactacaacatccagaaggagtcgacccttcaccttgtcctccgcctccgtggtggcatgcagatctttgtcaagactctgaccggcaagactatcacccttgaggtggagtcttctgacaccatcgacaacgtcaaggccaagatccaggacaaagagggcatccccccagaccagcagcgtctcatcttcgccggcaagcagctggaggatggcaggacccttgctgactacaacatccagaaggagtccaccctccaccttgtcctccgcctccgtggtggcatgcagatctttgtcaagacactgaccggcaagaccatcaccctcgaggtggaatcttctgacaccatcgacaacgtcaaggccaagatccaggacaaggagggcattcccccggaccagcagcgtctcatctttgccggcaagcagcttgaggacggcaggacccttgctgactacaacatccagaaggagtcaacgcttcaccttgtcctccgtctcaggggaggcatgcaaatcttcgtgaagactctgaccggcaagaccatcaccctcgaggtggagtcttctgataccatcgacaatgtcaaggccaagatccaggacaaggagggcattcccccggaccagcagcgcctcatctttgctggcaagcagctggaggatggcaggacccttgctgactacaacatccagaaggagtccaccctccaccttgtgctccgccttcgtggtggtatgcagatctttgtcaagaccctcacaggcaagaccatcaccctggaggttgagagctcggacaccatcgacaacgtcaaggccaagatccaggacaaggagggcatccccccagaccagcagcgtctcatcttcgccggcaagcagctcgaggatggccgcaccctcgccgactacaacatccagaaggagtctaccctccacctggtgcttcgtctccgtggtggtatgcagatcttcgtgaagaccttgactgggaagaccatcactttggaggttgagagctccgacaccattgataatgtgaaggccaagatccaggacaaggaggggattcccccagaccagcagcgtctgatcttcgctggcaagcagctggaggatggacgcaccctcgccgactacaacatccagaaggagtccaccctccacctggtgctccgcctccgtggtggtcagtaatcagccagtttggtggagctgccgatgtgcctggtcgtcccgagcctctgttcgtcaagtatttgtggtgctgatgtctacttgtgtctggtttaatggaccatcgagtccgtatgatatgttagttttatgaaacagtttcctgtgggacagcagtatgctttatgaataagttggatttgaacc

SEQ ID NO: 86 - DNA, 1971 bp, Oryza sativa
ggacaacttcctactcataggtgcttcgcaagtagcagcatccaagcactgaaaagtagtcagcatgtgagctttggagtgaaatctcttgtcttaaggaataaaggaaaaagattccgtcggaggctcggtgctctacaggttgtttgccaggactttccaagacctccactagaaaacacaataaactttttggaagctggacaactatcttcatttttcagaaacagtgaacaacccactaaaccattacaggtcgtgattgctggagcaggattagctggtttatcaacggcaaaatatctggcagatgctggtcataaacccatattgcttgaggcaagggatgttttgggtggaaagatagctgcttggaaggatgaagatggagattggtatgaaactgggcttcatatcttttttggagcttatcccaacatacagaacttgtttggcgagcttggtattaatgatcggttgcaatggaaggaacactccatgatatttgccatgccaaacaagccaggagaattcagccggtttgattttcctgaaacattgcctgcacccttaaatggaatatgggccatactaagaaacaatgaaatgctaacttggccagagaaggtgaagtttgctcttggacttttgccagcaatggttggtggccaagcttatgttgaagctcaagatggttttactgtttctgagtggatgaaaaagcagggtgttcctgatcgagtgaacgatgaggttttcattgcaatgtcaaaggcacttaatttcataaatcctgatgagttatccatgcagtgcattctgattgctttaaaccgatttcttcaggagaagcatggttctaagatggcattcttggatggtaatcctcctgaaaggttatgcatgcctattgttgaccatgttcgctctttgggtggtgaggttcggctgaattctcgtattcagaaaatagaacttaatcctgatggaacagtgaaacactttgcacttactgatggaactcaaataactggagatgcttatgtttttgcaacaccagttgatatcttgaagcttcttgtacctcaagagtggaaagaaatatcttatttcaagaagctggagaagttggtgggagttcctgttataaatgttcatatatggtttgatagaaaactgaagaacacatatgaccaccttcttttcagcaggagttcacttttaagtgtttatgcggacatgtcagtaacttgcaaggaatactatgatccaaaccgttcaatgctggagttggtctttgctcctgcagaggaatgggttggacggagtgacactgaaatcatcgaagcaactatgcaagagctagccaagctatttcctgatgaaattgctgctgatcagagtaaagcaaagattctgaagtatcatgttgtgaagacaccaagatctgtttacaagactatcccggactgtgaaccttgccgacctctgcaaagatcaccgattgaagggttctatctagctggtgactacacaaagcagaaatatttggcttcgatggagggtgcagttctatctgggaagctttgtgctcagtctgtagtggaggattataaaatgctatctcgtaggagcctgaaaagtctgcagtctgaagttcctgttgcctcctagttgtagtcaggactattcccaatggtgtgtgtgtcatcatcccctagtcagtttttttctatttagtgggtgcccaactctccaccaatttacacatgatggaacttgaaagatgcctattttggtcttatcatatttctgtaaagttgatttgtgactgagagctgatgccgatatgccatgctggagaaaaagaacattatgtaaaacgacctgcatagtaattcttagacttttgcaaaaggcaaaaggggtaaagcgaccttttttttctatgtgaagggattaagagacctt

SEQ ID NO: 87 - RNA, 250 nt, Artificial Sequence
  tRNA-gRNA-tRNA scheme
  misc_feature (78)..(97): n is a, c, g, or u
aacaaagcaccaguggucuagugguagaauaguacccugccacgguacagacccggguucgauucccggcuggugcannnnnnnnnnnnnnnnnnnnguuuuagagcuagaaauagcaaguuaaaauaaggcuaguccguuaucaacuugaaaaaguggcaccgagucggugcaacaaagcaccaguggucuagugguagaauaguacccugccacgguacagacccggguucgauucccggcuggugca

SEQ ID NO: 88 - RNA, 100 nt, Artificial Sequence
  gRNA from PTG gene
  misc_feature (1)..(20): n is a, c, g, or u
nnnnnnnnnnnnnnnnnnnnguuuuagagcuagaaauagcaaguuaaaauaaggcuaguccguuaucaacuugaaaaaguggcaccgagucggugcaaca

SEQ ID NO: 89 - RNA, 100 nt, Artificial Sequence
  gRNA from sgRNA gene
  misc_feature (2)..(20): n is a, c, g, or u
annnnnnnnnnnnnnnnnnnguuuuagagcuagaaauagcaaguuaaaauaaggcuaguccguuaucaacuugaaaaaguggcaccgagucggugcuuuu

SEQ ID NO: 90 - DNA, 27 bp, Oryza sativa
ccaaccattttccatggcgggaggttc

SEQ ID NO: 91 - DNA, 26 bp, Oryza sativa
ccaaccatttccatggcgggaggttc

SEQ ID NO: 92 - DNA, 26 bp, Oryza sativa
ttctccctccaggaggtggcaatcaa

SEQ ID NO: 93 - DNA, 61 bp, Oryza sativa
ttctccctcctaatctggaccaaagtgctgtccgcctacaacaagaggaggtggcaatcaa

SEQ ID NO: 94 - DNA, 29 bp, Oryza sativa
ttctcccctcctcaggaggtggcaatcaa

SEQ ID NO: 95 - DNA, 27 bp, Oryza sativa
gcggccggtactcatggacaccgacct

SEQ ID NO: 96 - DNA, 26 bp, Oryza sativa
gcggccggtatcatggacaccgacct

SEQ ID NO: 97 - DNA, 24 bp, Oryza sativa
atcaccctttggccaagcggacac

SEQ ID NO: 98 - DNA, 23 bp, Oryza sativa
atcaccctttgccaagcggacac

SEQ ID NO: 99 - DNA, 27 bp, Oryza sativa
atcaccctttcgatgccaagcggacac

SEQ ID NO: 100 - DNA, 31 bp, Oryza sativa
gcacggcggccggtatcatggacaccgacct

SEQ ID NO: 101 - DNA, 32 bp, Oryza sativa
cgcgtgccaaccatttgccatggcgggaggtt

SEQ ID NO: 102 - DNA, 85 bp, Oryza sativa
cgcacggcgccggtacctgctctacgacatcttcgggaacaagttcaacgacgtctacatcgccacggagctcatggacaccgac

SEQ ID NO: 103 - DNA, 87 bp, Oryza sativa
gtcggtgtccatgagctccgtggcgatgtagacgtcgttgaaacttgttcccgaagatgtcgtagagcaggtaccggccgccgtgcg

SEQ ID NO: 104 - DNA, 78 bp, Oryza sativa
gccaaccattttataccccggtgggccaccacccccacctatggagaacatccaggcgacgctgagccatggcgggag

SEQ ID NO: 105 - DNA, 78 bp, Oryza sativa
ctcccgccatggctcagcgtcgcctccatgttctccataggtgggggtggtggcccaccggggtataaaatggttggc

SEQ ID NO: 106 - DNA, 92 bp, Oryza sativa
cctccttctccctccttgaggcgaccgggttcgtttcttggctgtgcggttgtgaatgcgcagactcgtcaggaggtggcaatcaagaagat

SEQ ID NO: 107 - DNA, 92 bp, Oryza sativa
atcttcttgattgccacctcctgacgagtctgcgcattcacaaccgcacagccaagaaacgaacccggtcgcctcaaggagggagaaggagg

SEQ ID NO: 108 - DNA, 86 bp, Oryza sativa
tgatcaaccctttgattgacccgcacccgcatccctttccccattcgacaaccatatcgatgccaagcggacactgagagaaatca

SEQ ID NO: 109 - DNA, 83 bp, Oryza sativa
tgatttctcagtgtccgcttggcatcgatatggttgtcgaatggggaaagggatgcgggtgcgggtcaatcaaagggtgatca

SEQ ID NO: 110 - DNA, 100 bp, Artificial Sequence
  Vector
aaggaatctttaaacatgatttaaaagagttgtgcagatgatccgtggcaggagaccgaggtctcggttttagagctagaaaccgagtcggtgctttttt

SEQ ID NO: 111 - DNA, 100 bp, Artificial Sequence
  Vector
aaaaaagcaccgactcggtttctagctctaaaaccgagacctcggtctcctgccacggatcatctgcacaactcttttaaatcatgtttaaagattcctt

SEQ ID NO: 112 - DNA, 44 bp, Oryza sativa
agtggcaccgagtcggtgctttaagatgtcgtagagcaggtacg

SEQ ID NO: 113 - DNA, 42 bp, Oryza sativa
agtggcaccgagtcggtgctaagatgtcgtagagcaggtacg

SEQ ID NO: 114 - DNA, 43 bp, Oryza sativa
agtggcaccgagtcggtgcttaagatgtcgtagagcaggtacg

SEQ ID NO: 115 - DNA, 46 bp, Oryza sativa
gtggcaccgagtcggtgctttttttagatgtcgtagagcaggtacg

SEQ ID NO: 116 - DNA, 37 bp, Oryza sativa
ggcaccgagtcggtgctttacatcgccacggagctca

SEQ ID NO: 117 - DNA, 44 bp, Oryza sativa
aagtggcaccgagtcggtgctttctacatcgccacggagctcag

SEQ ID NO: 118 - DNA, 46 bp, Oryza sativa
agtggcaccgagtcggtgcaaagatgtcgtagagcaggtacaatcg

SEQ ID NO: 119 - DNA, 47 bp, Oryza sativa
aaaagtggcaccgagtcggtgcaatctacatcgccacggagctcagt

SEQ ID NO: 120 - DNA, 67 bp, Oryza sativa
cgcgtgccaaccatttataccccggtgggccacatccaggcgacgctgaaaccatggcgggaggttc

SEQ ID NO: 121 - DNA, 63 bp, Oryza sativa
cgcgtgccaaccatttataccccggtgggccacatccaggcgacgctccatggcgggaggttc

SEQ ID NO: 122 - DNA, 65 bp, Oryza sativa
cgcgtgccaaccatttataccccggtgggccacatccaggcgacgctgaccatggcgggaggttc

SEQ ID NO: 123 - DNA, 39 bp, Oryza sativa
tcctccttctccctcctgaggcgaccgggttcgaatgcg

SEQ ID NO: 124 - DNA, 68 bp, Oryza sativa
tcctccttctccctcctttgaggcgaccgggttcgaatgcgcagactcgtctaggaggtggcaatcaa

SEQ ID NO: 125 - DNA, 56 bp, Oryza sativa
tcctccttaggcgaccgggttcgaatgcgcagactcgtctaggaggtggcaatcaa

SEQ ID NO: 126 - DNA, 61 bp, Oryza sativa
cgcacggcggccggtatacgacatcttctacatcgccacggagcatcatggacaccgacct

SEQ ID NO: 127 - DNA, 52 bp, Oryza sativa
cgcacggcggccggtattctacatcgccacggagcttcatggacaccgacct

SEQ ID NO: 128 - DNA, 32 bp, Oryza sativa
cgcacggcggccggtatcatggacaccgacct

SEQ ID NO: 129 - DNA, 59 bp, Oryza sativa
ggtgtgatcacccttttacccgcacccgccattcgacaaccatattgccaagcggacac

SEQ ID NO: 130 - DNA, 58 bp, Oryza sativa
ggtgtgatcaccctttatgacccgcacccgccattcgacaaccataccaagcggacac

SEQ ID NO: 131 - DNA, 64 bp, Oryza sativa
ggtgtgatcaccctttagacccgcacccgccattcgacaaccatatacgatgccaagcggacac

SEQ ID NO: 132 - DNA, 76 bp, Oryza sativa
gccatgccaaacaagccaggagaattcagccggtttgaaaatcctgatgagttatccatgcagtgcattctgattg

SEQ ID NO: 133 - DNA, 26 bp, Oryza sativa
ccatgccaaacaagccagccggttga

SEQ ID NO: 134 - DNA, 31 bp, Oryza sativa
aaatcctgatatccatgcagtgcattctgat

SEQ ID NO: 135 - DNA, 50 bp, Oryza sativa
cgcgtgccaaccatttataccccggtggccacatccatggcgggaggttc

SEQ ID NO: 136 - DNA, 62 bp, Oryza sativa
cgcgtgccaaccaggggaccccggtgggccacatccaggcgacgctgaatggcgggaggttc

SEQ ID NO: 137 - DNA, 68 bp, Oryza sativa
cgcgtgccaaccaaccattttataccccggtgggccacatccaggcgacgctccatggcgggaggttc

SEQ ID NO: 138 - DNA, 65 bp, Oryza sativa
cgcgtgccaaccatttatataccccggtgggccacatccaggcgacgctccatggcgggaggttc

SEQ ID NO: 139 - DNA, 64 bp, Oryza sativa
cgcgtgccaaccattttatatcccggtgggccacatccaggcgacgctccatggcgggaggttc

SEQ ID NO: 140 - DNA, 63 bp, Oryza sativa
cgcgtgccaaccatttgtgccccggtgggccacatccaggcgacgctccatggcgggaggttc

SEQ ID NO: 141 - DNA, 66 bp, Oryza sativa
tcctccttctccctccgaggcgaccgggttcgaatgcgcagactcgtcaaaggaggtggcaatcaa

SEQ ID NO: 142 - DNA, 68 bp, Oryza sativa; identical to SEQ ID NO: 124

SEQ ID NO: 143 - DNA, 68 bp, Oryza sativa
tcctccttctccctcctttgaggcgaccgggttcgaatgcgcagactcgtccaggaggtggcaatcaa

SEQ ID NO: 144 - DNA, 54 bp, Oryza sativa
tcctccttaggcgaccgggttcgaatgcgcagactcgtcggaggtggcaatcaa

SEQ ID NO: 145 - DNA, 54 bp, Oryza sativa; identical to SEQ ID NO: 144

SEQ ID NO: 146 - DNA, 71 bp, Oryza sativa
cgcacggcggccggtatcctgctctacgacatcttctctacatcgccacggagcctcatggacaccgacct

SEQ ID NO: 147 - DNA, 57 bp, Oryza sativa
cgcacggcggccgcttctctacgacatcttctctacatcgctcatggacaccgacct

SEQ ID NO: 148 - DNA, 56 bp, Oryza sativa
cgcacggcggccgctatctacgacatcttctctacatcgctcatggacaccgacct

SEQ ID NO: 149 - DNA, 65 bp, Oryza sativa
cgcacggcggccgctatctacgacatcttctctacatcgccacggagcttcatggacaccgacct

SEQ ID NO: 150 - DNA, 58 bp, Oryza sativa
ggtgtgatcaccttgacccgcagggcgattcgacaaccatccgatgccaagcggacac

SEQ ID NO: 151 - DNA, 26 bp, Oryza sativa
acccgcacccgctgccaagcggacac

SEQ ID NO: 152 - DNA, 58 bp, Oryza sativa
ggtgtgatcaccctttaacccgcacccgcattcgacaaccatattgccaagcggacac

SEQ ID NO: 153 - DNA, 53 bp, Oryza sativa
ggtgtgatcaccctttacacccgcattcgacaaccatattgccaagcggacac

SEQ ID NO: 154 - DNA, 53 bp, Oryza sativa; identical to SEQ ID NO: 153

SEQ ID NO: 155 - DNA, 57 bp, Oryza sativa
ggtgtgatcaccctttacacccgcattcgacaaccatatacgatgccaagcggacac

SEQ ID NO: 156 - protein, 55 aa, Oryza sativa
MDAGAQPPDTEMAEAGGGQQPPAAAAAAGAGAGAGMMENIHGGRFIQYNIFGNVF

SEQ ID NO: 157 - protein, 59 aa, Oryza sativa
MDAGAQPPDTEMAEAGGGQQPPAAAAAAGAGAGAGMMENIQATLHGGRFIQYNIFGNVF

SEQ ID NO: 158 - protein, 59 aa, Oryza sativa
MDAGAQPPDTEMAEAGGGQQPPAAAAAAGAGAGAGMMENIQATLNGGRFIQYNIFGNVF

SEQ ID NO: 159 - protein, 21 aa, Oryza sativa
MDGAPVAEFRPTMTHGGRYPA

SEQ ID NO: 160 - protein, 19 aa, Oryza sativa
MDGAPVAEFRPTMTHGGRY

SEQ ID NO: 161 - protein, 19 aa, Oryza sativa
MDGAPVAEFRPTMTHGGRY

SEQ ID NO: 162 - protein, 19 aa, Oryza sativa
MDGAPVAEFRPTMTHGGRF

SEQ ID NO: 163 - protein, 31 aa, Oryza sativa
GCACGGCGGCCGGTATCATGGACACCGACCT

SEQ ID NO: 164 - DNA, 20 bp, Artificial Sequence
  sg1 target Human HDAC1
gtaagaccaccgcactaggc

SEQ ID NO: 165 - DNA, 20 bp, Artificial Sequence
  sg2 target Human HDAC1
gccctgcagctattaccatt

SEQ ID NO: 166 - DNA, 20 bp, Artificial Sequence
  sg1 target Human HDAC2
gtattttaggatattggtgc

SEQ ID NO: 167 - DNA, 20 bp, Artificial Sequence
  sg2 target Human HDAC2
tgtttcaatctaacagtcaa

SEQ ID NO: 168 - DNA, 20 bp, Artificial Sequence
  sg1 target human HDAC3
gagcagaactcaaagagccc

SEQ ID NO: 169 - DNA, 20 bp, Artificial Sequence
  sg2 target human HDAC3
gctcaagtaagtagcccagg

SEQ ID NO: 170 - DNA, 20 bp, Artificial Sequence
  sg1 target human HDAC4
gagctcctgaatacgtcgca

SEQ ID NO: 171 - DNA, 20 bp, Artificial Sequence
  sg2 target human HDAC4
gctcctttgccgtccccgag

SEQ ID NO: 172 - DNA, 20 bp, Artificial Sequence
  sg1 target human HDAC6
cgactggcagcaggacgtgc

SEQ ID NO: 173 - DNA, 20 bp, Artificial Sequence
  sg2 target human HDAC6
caagctgatcctgtctctgg

SEQ ID NO: 174 - DNA, 20 bp, Artificial Sequence
  Primer: Genotyping of MPK1
cctcgtgtttggtgttgctg

SEQ ID NO: 175 - DNA, 20 bp, Artificial Sequence
  Primer: Genotyping of MPK2
tgcgcctaaaaatcgagggt

SEQ ID NO: 176 - DNA, 21 bp, Artificial Sequence
  Primer: Genotyping MPK2
tttgggaagcatgtatgaagc

SEQ ID NO: 177 - DNA, 20 bp, Artificial Sequence
  Primer: Gentoyping MPK2
tatgccagccaatgagccaa

SEQ ID NO: 178 - DNA, 21 bp, Artificial Sequence
  Genotyping of MPK5
gccaccttccttcctcatccg

SEQ ID NO: 179 - DNA, 20 bp, Artificial Sequence
  Genotyping of MPK5
actccgtcatcatgtcgctc

SEQ ID NO: 180 - DNA, 21 bp, Artificial Sequence
  Genotyping of MPK6
ttgacgccccaacataaataa

SEQ ID NO: 181 - DNA, 18 bp, Artificial Sequence
  Genotyping of MPK6
tgttgctgccgcttttct

SEQ ID NO: 182 - DNA, 41 bp, Artificial Sequence; identical to SEQ ID NO: 41
  Detection of U3:PTG

SEQ ID NO: 183 - DNA, 37 bp, Artificial Sequence; identical to SEQ ID NO: 42
  Detection of U3:PTG

SEQ ID NO: 184 - DNA, 20 bp, Artificial Sequence
  Detection of Cas9
gcttgtgcgtttcgatttga

SEQ ID NO: 185 - DNA, 20 bp, Artificial Sequence
  Detection of Cas9
ccgctcgtgcttcttatcct

SEQ ID NO: 186 - DNA, 19 bp, Artificial Sequence
  Control for DNA quality
cgctgccactctccactga

SEQ ID NO: 187 - DNA, 20 bp, Artificial Sequence
  Control for DNA quality
agctgcttccactcgttcca

SEQ ID NO: 188 - DNA, 77 bp, Artificial Sequence
  tRNA1 for PTG7
aataaagcaccagtggtctagtggtagaatagtaccctgccacggtacagacccgggttcgattcccggctggtgca

SEQ ID NO: 189 - DNA, 77 bp, Artificial Sequence; identical to SEQ ID NO: 13
  tRNA used for PTG10